European Patent Application EP 4 640 707 A1, published October 29, 2025. Title: Anti-cMet 抗体、抗体药物偶联物及其制备方法和用途. Applicant: 苏州宜联生物医药有限公司. Application WO. The sequence listing filed with the application follows.

SEQUENCE LISTING (61 sequences)

SEQ ID NO: 1 - protein, 110 aa, synthetic construct
IVMTQSPASLPVSLGQRATISCRASESVDDYGVSFVNWFQQKPGQPPKLLIYTASVQESGVPARFSGSGSGTDFSLNIHPLEEDDTAMYFCQQSKEIPPTFGGGTKLEIK

SEQ ID NO: 2 - protein, 116 aa, synthetic construct
EVRLEESGGGFVQPGGSMKISCVASGFTFSNYWMNWVRQSPEKGLEWVAQIRLKSLNYATHYAESVKGRFTISRDDSRNSVYLQMNNLRAEDAGIYYCTEEGFAYWGRGTLVTVSA

SEQ ID NO: 3 - protein, 107 aa, synthetic construct
DIQMTQSPPSLSASVGETVTITCGASENIYGALNWYQRKQGKSPQLLIYGATNLAAGMSSRFSGSGSGRQFSLKISSLHPDDVATYYCQNVLSEPLTFGAGTKLELK

SEQ ID NO: 4 - protein, 117 aa, synthetic construct
QIQLQQSGPELVKPGASVKISCKASGYTFTDYYLNWVRQRPGQGLEWIGWIFPGSGNTKYIEKFKGKATLTVDTSSSTAYMLLSSLTSEDSAVYFCAGGDYGGFTYWGQGTLVAVSA

SEQ ID NO: 5 - protein, 112 aa, synthetic construct
NIMMTQSPSSLAVSAGEKVTMNCKSSQSVLYFSNQKNCLAWYQQKPGQSPKLLIYWASTRESGVPDRFTGSGSGTDFTLTISSVQADDLAVYYCQQYLSSLTFGAGTKLELK

SEQ ID NO: 6 - protein, 121 aa, synthetic construct
QVHLQQSGAELARPGASVKMSCKASGYTFISYTIHWVKQSPGQGLEWIGYINPSSGYAKNNPKFQDKATLTADTSSTTAYIQLSSLTSEDSAVYYCTRPYGDFVDWYFDVWGTGTTVTVSS

SEQ ID NO: 7 - protein, 110 aa, synthetic construct
IVMTQSPASLPVSLGQRATISCRASESVDDYGVSFVNWFQQKPGQPPKLLIYTASVQESGVPARFSGSGSGTDFRLNIHPLEEDDTAMYFCQQSKEIPPTFGGGTKLEIK

SEQ ID NO: 8 - protein, 116 aa, synthetic construct
EVRLEDSGGGFVQPGGSMKISCVASGFTFSNYWMNWVRQSPEKGLEWVAQIRLKSLNYATHYAESVKGRFTISRDDSRNSVYLQMNNLRAEDAGIYYCTEEGFAYWGRGTLVTVSA

SEQ ID NO: 9 - protein, 111 aa, synthetic construct
DIVMTQSPSSLAVSLGQRATINCRASESVDDYGVSFVNWFQQKPGQPPKLLIYTASVQESGVPDRFSGSGSGTDFTLTISSLQAEDVAVYFCQQSKEIPPTFGQGTKVEIK

SEQ ID NO: 10 - protein, 116 aa, synthetic construct
EVQLVQSGGGLVQPGGSLRLSCAASGFTFSNYWMNWVRQAPGKGLEWVAQIRLKSLNYATHYAQSVKGRFTISRDDAKNSVYLQMNSLRAEDTAVYYCTEEGFAYWGQGTLVTVSS

SEQ ID NO: 11 - protein, 107 aa, synthetic construct
DIQMTQSPSSLSASVGDRVTITCGASENIYGALNWYQQKPGKAPKLLIYGATNLAAGVPSRFSGSGSGRDFTLTISSLQPEDFATYYCQNVLSEPLTFGQGTKVEIK

SEQ ID NO: 12 - protein, 117 aa, synthetic construct
QIQLVQSGAEVKKPGASVKVSCKASGYTFTDYYLNWVRQAPGQGLEWMGWIFPGSGNTKYSQKFQGRVTLTVDTSASTAYMELSSLRSEDTAVYYCAGGDYGGFTYWGQGTLVTVSS

SEQ ID NO: 13 - protein, 8 aa, synthetic construct
GFTFSNYW

SEQ ID NO: 14 - protein, 10 aa, synthetic construct
IRLKSLNYAT

SEQ ID NO: 15 - protein, 7 aa, synthetic construct
TEEGFAY

SEQ ID NO: 16 - protein, 5 aa, synthetic construct
NYWMN

SEQ ID NO: 17 - protein, 19 aa, synthetic construct
QIRLKSLNYATHYAESVKG

SEQ ID NO: 18 - protein, 19 aa, synthetic construct
QIRLKSLNYATHYAQSVKG

SEQ ID NO: 19 - protein, 5 aa, synthetic construct
EGFAY

SEQ ID NO: 20 - protein, 10 aa, synthetic construct
ESVDDYGVSF

SEQ ID NO: 21 - skipped

SEQ ID NO: 22 - protein, 9 aa, synthetic construct
QQSKEIPPT

SEQ ID NO: 23 - protein, 15 aa, synthetic construct
RASESVDDYGVSFVN

SEQ ID NO: 24 - protein, 7 aa, synthetic construct
TASVQES

SEQ ID NO: 25 - protein, 7 aa, synthetic construct
GFTFSNY

SEQ ID NO: 26 - protein, 8 aa, synthetic construct
GYTFTDYY

SEQ ID NO: 27 - protein, 8 aa, synthetic construct
IFPGSGNT

SEQ ID NO: 28 - protein, 10 aa, synthetic construct
AGGDYGGFTY

SEQ ID NO: 29 - protein, 5 aa, synthetic construct
DYYLN

SEQ ID NO: 30 - protein, 17 aa, synthetic construct
WIFPGSGNTKYIEKFKG

SEQ ID NO: 31 - protein, 17 aa, synthetic construct
WIFPGSGNTKYSQKFQG

SEQ ID NO: 32 - protein, 8 aa, synthetic construct
GDYGGFTY

SEQ ID NO: 33 - protein, 6 aa, synthetic construct
ENIYGA

SEQ ID NO: 34 - skipped

SEQ ID NO: 35 - protein, 9 aa, synthetic construct
QNVLSEPLT

SEQ ID NO: 36 - protein, 11 aa, synthetic construct
GASENIYGALN

SEQ ID NO: 37 - protein, 7 aa, synthetic construct
GATNLAA

SEQ ID NO: 38 - protein, 19 aa, synthetic construct
  VARIANT 15: note = x can be any amino acid, e.g, E or Q.
QIRLKSLNYATHYAXSVKG

SEQ ID NO: 39 - protein, 8 aa, synthetic construct
GYTFISYT

SEQ ID NO: 40 - protein, 8 aa, synthetic construct
INPSSGYA

SEQ ID NO: 41 - protein, 14 aa, synthetic construct
TRPYGDFVDWYFDV

SEQ ID NO: 42 - protein, 5 aa, synthetic construct
SYTIH

SEQ ID NO: 43 - protein, 17 aa, synthetic construct
YINPSSGYAKNNPKFQD

SEQ ID NO: 44 - protein, 12 aa, synthetic construct
PYGDFVDWYFDV

SEQ ID NO: 45 - protein, 12 aa, synthetic construct
QSVLYFSNQKNC

SEQ ID NO: 46 - skipped

SEQ ID NO: 47 - protein, 8 aa, synthetic construct
QQYLSSLT

SEQ ID NO: 48 - protein, 17 aa, synthetic construct
KSSQSVLYFSNQKNCLA

SEQ ID NO: 49 - protein, 7 aa, synthetic construct
WASTRES

SEQ ID NO: 50 - protein, 8 aa, synthetic construct
QQYLSSLT

SEQ ID NO: 51 - protein, 330 aa, synthetic construct [sequence omitted]

SEQ ID NO: 52 - protein, 107 aa, synthetic construct [sequence omitted]

SEQ ID NO: 53 - protein, 8 aa, synthetic construct
RLKSLNYA

SEQ ID NO: 54 - protein, 7 aa, synthetic construct
GYTFTDY

SEQ ID NO: 55 - protein, 6 aa, synthetic construct
FPGSGN

SEQ ID NO: 56 - protein, 446 aa, synthetic construct
EVQLVQSGGGLVQPGGSLRLSCAASGFTFSNYWMNWVRQAPGKGLEWVAQIRLKSLNYATHYAQSVKGRFTISRDDAKNSVYLQMNSLRAEDTAVYYCTEEGFAYWGQGTLVTVSSASTKGPSVFPLAPSSKSTSGGTAALGCLVKDYFPEPVTVSWNSGALTSGVHTFPAVLQSSGLYSLSSVVTVPSSSLGTQTYICNVNHKPSNTKVDKKVEPKSCDKTHTCPPCPAPELLGGPSVFLFPPKPKDTLMISRTPEVTCVVVDVSHEDPEVKFNWYVDGVEVHNAKTKPREEQYNSTYRVVSVLTVLHQDWLNGKEYKCKVSNKALPAPIEKTISKAKGQPREPQVYTLPPSRDELTKNQVSLTCLVKGFYPSDIAVEWESNGQPENNYKTTPPVLDSDGSFFLYSKLTVDKSRWQQGNVFSCSVMHEALHNHYTQKSLSLSPGK

SEQ ID NO: 57 - protein, 218 aa, synthetic construct
DIVMTQSPSSLAVSLGQRATINCRASESVDDYGVSFVNWFQQKPGQPPKLLIYTASVQESGVPDRFSGSGSGTDFTLTISSLQAEDVAVYFCQQSKEIPPTFGQGTKVEIKRTVAAPSVFIFPPSDEQLKSGTASVVCLLNNFYPREAKVQWKVDNALQSGNSQESVTEQDSKDSTYSLSSTLTLSKADYEKHKVYACEVTHQGLSSPVTKSFNRGEC

SEQ ID NO: 58 - protein, 447 aa, synthetic construct
QIQLVQSGAEVKKPGASVKVSCKASGYTFTDYYLNWVRQAPGQGLEWMGWIFPGSGNTKYSQKFQGRVTLTVDTSASTAYMELSSLRSEDTAVYYCAGGDYGGFTYWGQGTLVTVSSASTKGPSVFPLAPSSKSTSGGTAALGCLVKDYFPEPVTVSWNSGALTSGVHTFPAVLQSSGLYSLSSVVTVPSSSLGTQTYICNVNHKPSNTKVDKKVEPKSCDKTHTCPPCPAPELLGGPSVFLFPPKPKDTLMISRTPEVTCVVVDVSHEDPEVKFNWYVDGVEVHNAKTKPREEQYNSTYRVVSVLTVLHQDWLNGKEYKCKVSNKALPAPIEKTISKAKGQPREPQVYTLPPSRDELTKNQVSLTCLVKGFYPSDIAVEWESNGQPENNYKTTPPVLDSDGSFFLYSKLTVDKSRWQQGNVFSCSVMHEALHNHYTQKSLSLSPGK

SEQ ID NO: 59 - protein, 214 aa, synthetic construct
DIQMTQSPSSLSASVGDRVTITCGASENIYGALNWYQQKPGKAPKLLIYGATNLAAGVPSRFSGSGSGRDFTLTISSLQPEDFATYYCQNVLSEPLTFGQGTKVEIKRTVAAPSVFIFPPSDEQLKSGTASVVCLLNNFYPREAKVQWKVDNALQSGNSQESVTEQDSKDSTYSLSSTLTLSKADYEKHKVYACEVTHQGLSSPVTKSFNRGEC

SEQ ID NO: 60 - protein, 6 aa, synthetic construct
NPSSGY

SEQ ID NO: 61 - protein, 17 aa, synthetic construct
  VARIANT 12: note = x can be any amino acid, e.g., I or S.
  VARIANT 13: note = x can be any amino acid, e.g., E or Q.
  VARIANT 16: note = x can be any amino acid, e.g., K or Q.
WIFPGSGNTKYXXKFXG